European Patent Application EP 4 197 537 A1, published June 21, 2023. Title: A Composition for Preventing or Treating Hepatic Fibrosis Comprising Triazole Derivatives as Active Ingredients. Applicant: Industry-Academic Cooperation Foundation Yonsei University. The sequence listing filed with the application follows.

SEQUENCE LISTING (8 sequences)

SEQ ID NO: 1 - DNA, 20 bp, Artificial Sequence
  COL1A1 F primer
gcttcacctacagcaccctt

SEQ ID NO: 2 - DNA, 20 bp, Artificial Sequence
  COL1A1 R primer
gtccgaattcctggtctggg

SEQ ID NO: 3 - DNA, 23 bp, Artificial Sequence
  CCL2 F primer
taaaaaacctggatcggaaccaa

SEQ ID NO: 4 - DNA, 23 bp, Artificial Sequence
  CCL2 R primer
gcattagcttcagatttacgggt

SEQ ID NO: 5 - DNA, 20 bp, Artificial Sequence
  TGF-beta F primer
cctgcaagaccatcgacatg

SEQ ID NO: 6 - DNA, 20 bp, Artificial Sequence
  TGF-beta R primer
tgttgtacaaagcgagcacc

SEQ ID NO: 7 - DNA, 20 bp, Artificial Sequence
  F4/80 F primer
cgtcagccgatttgctatct

SEQ ID NO: 8 - DNA, 20 bp, Artificial Sequence
  F4/80 R primer
cggactccgcaaagtctaag